European Patent Application EP 4 309 500 A1, published January 24, 2024. Title: PEROXIDASE BASED BIOCONTROL AGENTS. Applicant: Acies Bio d.o.o. Application EP. The sequence listing filed with the application follows.

SEQUENCE LISTING (28 sequences)

SEQ ID NO: 1 - protein, 659 aa, Hydrocoleum sp.
MDDNYENNNSIQQAFDFSENEQTLLSNINGLGVALDNDFYEIEATEGSLDIFVELTFNHNEGNLDLFLFDSTGNEIASSNSLDDNEIIDFTVDKAGTYYIQVTSGDGTFSGNTYDLFWDDVIAENTFRTINGLNNNLQNPEFGSATEKGTRYTQLLRLGPEAYQDELSEPRGGGLTTPLELPSAREVSNAIADQGEQSIANDFKLSDWFWQWGQFIDHDISLTEADTSGDSFPIPVPTGDPDFDPFGTGTQTIPLTRSIFDPATGTTNPREQINEITAFLDGSMVYGSDEATALSLRANDGTGKLATSIGPDGEILLPTDSDGNFLAGDIRVNEQLGLISVHTLFVREHNRLAQKTADVLDNGKGRKANKLNELFEESGLSRGDFIYESARRLVGAEIQTITYNEFLPFLLGKNVLDKYTGYDETVDPGIFTEFSTGVFRFGHTMLSPQLLQVEEDGSYEAVALRDAFFQPGKIMEDGVDSLLKGLESQQAQEVDNLLIDDVRNFLFGRPGAGGFDLASLNIQRGRENGVADINTFRNAIGLSPYTDFDELTGGDSELAAKFASVYDSIDDVDLWIGGLAEQDVNGGVVGETISAIIIEQFSNLRDGDRFYFENDQYLKELKGILDKNIDKVSLANIIEDNSDVQIVGSAFTVNNPIVV

SEQ ID NO: 2 - DNA, 1980 bp, synthetic construct
  source 1..1980: mol_type = other DNA
atggatgataattacgaaaacaataattccattcagcaggcgtttgattttagcgagaatgaacaaacgcttctttccaatattaatgggcttggcgttgcccttgataacgatttttatgaaattgaagcgacagaaggcagtctggatatttttgtcgaattaacatttaaccataatgagggaaaccttgatctttttcttttcgattcgacaggcaacgaaattgcctcatctaacagtctcgatgacaatgaaattattgactttactgtagacaaggccggcacatattatattcaagtgacgagcggggatggcacgttttcgggcaacacatatgatctgttctgggatgacgtgatcgcagaaaatacatttcgtacgattaacggacttaataacaatttgcaaaatcccgaatttggatcagcgaccgagaaaggtaccaggtatacacaactacttagacttggaccagaagcttatcaggatgaactgagcgaaccgcgcggaggtggcttaaccacacccctggagttgccgtctgcccgagaggtgtctaacgctatcgccgatcagggcgaacaatccatcgcgaacgattttaaattgtcagattggttctggcaatggggacagtttattgatcacgacatcagcctcacagaagcggatacctcaggtgattcctttccgatcccagttccgacaggtgacccggatttcgatccattcggtactggaacgcagacaatcccgttgactcgctcaatttttgatcctgctacaggtacaacaaaccctcgtgaacagattaacgagataacggctttcttggatggttccatggtatacggcagcgacgaagcaacagcactgagccttagagcgaatgatggcactggaaaattggcaacatctatcggcccggatggggaaattctgctcccgacagactctgatgggaattttttggcaggtgatattagagttaacgaacaactaggtttaatctcagtacatacattgtttgttcgggaacacaatagactggcgcaaaaaaccgcggacgtcttagataacggcaaagggcgaaaggccaacaaacttaatgaactgttcgaagaatcaggcttgagccgaggagattttatctacgaatcagctaggcgtctggttggagcggaaattcaaacaatcacatataacgaatttcttccttttcttttagggaaaaatgtcctcgataagtacacagggtacgacgaaacggtcgatcctggcatattcacagaatttagcacaggcgtttttcgatttgggcatacgatgttatcaccacagctgttacaagtggaggaagatggctcgtatgaagcagttgctttaagagatgctttttttcagccaggcaaaattatggaagatggggttgattcactcctgaaaggactggagagccaacaggcacaagaagtggacaatcttctgattgacgacgttagaaacttcttatttgggcggccaggagcgggagggttcgacttagcatccttgaatatacaacgcgggcgcgagaatggagttgcagatattaacacgtttagaaacgccatcggtcttagcccgtatacagatttcgatgagcttaccggaggagattcagaattggcagcgaaattcgcttccgtctatgattcgattgatgatgtagacttgtggataggaggccttgctgaacaggatgtaaatggcggtgttgtgggggaaacaatctcagccattattatcgaacaatttagcaatctccgcgacggcgaccgtttctatttcgaaaatgatcaataccttaaagagttaaagggaattcttgataaaaacattgataaagttagcctcgctaacatcattgaagataactccgatgtgcaaattgtggggtccgcgttcacagtcaacaatccgattgtagtgtaa

SEQ ID NO: 3 - DNA, 42 bp, synthetic construct
  source 1..42: mol_type = other DNA
catcatcaccaccaccattaactgcaggcatgcaagcttggc

SEQ ID NO: 4 - DNA, 20 bp, synthetic construct
  source 1..20: mol_type = other DNA
catatgtgcaccggccgcag

SEQ ID NO: 5 - DNA, 47 bp, synthetic construct
  source 1..47: mol_type = other DNA
ctgcggccggtgcacatatggatgataattacgaaaacaataattcc

SEQ ID NO: 6 - DNA, 51 bp, synthetic construct
  source 1..51: mol_type = other DNA
cagttaatggtggtggtgatgatgcactacaatcggattgttgactgtgaa

SEQ ID NO: 7 - DNA, 1661 bp, synthetic construct
  source 1..1661: mol_type = other DNA
cggccggtgcacatatgggtgtctactatattaaagtgaagagcattggtaaaccgggaaactcatatgaccttgtatgggatgatatcgttcctattgagtttcggtctattgaagggctgaacaacaatttggtcaatccggactggggcacaccggactcacagcttatccgtctgagcgaatcagcatacaacgacgaaattagcgagcctcgcggcggcgatccatcttctttagttagccctcgggaagtctcaaacacaattttcgatcagagcgaatcaatccctaatgagacgggcgtatctgactggttttggcaatggggccagtttatcgatcatgacatggatttgaccccgggaacatctggtgaatcatttaatatcagcgtgccactgggtgatccatcatttgacccgtttaatagcggaacccaagaaatcccgctgaccagatcaatctatgattttgatactggaattgattctccgcgtgaacaaatcaatgagatcacggcgtatattgacggatctaatgtgtatggaagcgattcagagcgcgccgaagctttgagaacgaatgatgggacaggaaaactgaagacgtctgtaagcgaatctggtgaagtcctgttaccgttcaacacagatggacttgataatgacaatccattcggaattgcaaacgattcaatttttgtagctggcgacgttcgggcgaatgaacaagttgggttaactgccacacatacattatttgttcgggaacataaccgtctggccgatgatatcgcgacccgcctggataatggtgatgcggaattgttagacctttttgcagagagcggactgtcagaaggcgatttcatctacgaaagcgctagacgcatcgttggggcagagattcaagcaattacgtacaatgaattcgttccgctgcttgtaggatcaaacgctcttgacggatatgacggctataatgtaacagtagatagcgggattagcaacgaattttctacggcagcctttagatttggacacactatgctgagccctacgcttcaaaatgggacgaatgaaggtctgagcctgcgcgatacctttttcaatccggatttagtggtcgaaggcggcgtagattctttgttattggggcttgcatctcaagaagctcaggaagtcgacactcaagtgattgatgatgtgcgtaactttttatttggtgcgcctggttctggtggccttgatcttgttagcttaaacatccagcgtggccgggatcatgggttgccgtcatatactgaagttagagaagagctgggattagatccgattacaaatttcggcgagatcacaagcgatccaattgtccaggcccaacttgagtcagcttatacagacgtcgacaatattgatttgtgggttggcggcttagcagaagaccacgtcaacggaagcttgtttggcgagacatttcaggtgattgtcgtggaccagtttactcgccttagagacggcgatagattctactatgagaacgataatttactttcagtgcttgcgcctgacgttgcggaaacgacattgtctgatgtgattgtggccaacagcgctatctcttcaatccagtcaaatgcgttcctggtctaactgcag

SEQ ID NO: 8 - DNA, 1977 bp, synthetic construct
  source 1..1977: mol_type = other DNA
atggacgataattacgaaaacaataatagtatccaacaagcttttgatttttcagagaatgaacagactcttctgagcaacattaatgggctgggagttgctttagataatgacttttatgaaattgaagccacagaaggctctttagatatctttgtcgagttaacctttaaccataatgaaggaaatcttgatttatttctctttgattcaacaggaaatgaaattgcctcttcaaattctctagatgataatgaaataattgattttactgttgacaaagcaggaacttattatatccaagttacttcaggggatggtactttttcagggaatacctatgatttgttctgggatgatgttattgccgaaaatacctttcgcactattaatggtttaaataataatcttcaaaaccctgaatttggtagtgcaacagaaaaaggcactcgatacactcaattattacgcttaggtcctgaagcttaccaagatgaattatctgaaccaagaggtggtggactaactacgccccttgaacttcctagtgcgcgggaagtcagtaatgcgatcgccgatcaaggagaacaatctattgccaacgactttaaactttctgactggttttggcagtggggacaatttatcgatcatgacatcagtttaacagaagccgacacttcaggggactcatttcctattccagttcctacaggcgatccagattttgatccttttggcacaggaactcaaaccatacccttaactcgttctattttcgatcctgccaccggaaccacaaacccccgtgaacagattaacgaaattacagcgtttcttgatggttctatggtttatggttccgatgaagcaacggccctttctttgcgagctaatgatggcactggaaaactagccaccagcatcggtcctgatggggagattttactgcctactgatagtgatggtaactttcttgccggggatatccgtgttaatgaacaattaggcttaatttctgttcacaccctttttgttagagaacataaccgcttggcacaaaaaactgctgatgttttagacaatgggaagggaagaaaagcaaacaaactgaatgaactgtttgaagagtctgggttaagtcgtggtgactttatctatgaatcagcccgccgtttagttggggcagaaattcagaccattacctataatgaatttttacccttcctcttaggaaagaatgttcttgataagtatacgggttatgatgaaaccgtcgatcctggtattttcactgaattctccactggtgttttccgctttggtcataccatgctttctcctcaactcttacaagtggaagaggatggaagctatgaagcggttgctctacgggatgctttctttcaacctggcaaaattatggaggatggagttgattctttattgaaagggttagaatcccaacaagcccaagaagttgataatttactgattgatgatgttcgtaacttcttgtttggtcgtcctggggctggtggttttgacttagcctctcttaatattcaacggggacgggagaatggtgtagctgatattaatacatttcgtaatgctatcggtttatcgccttatacagactttgatgaattaacaggaggagacagcgagcttgctgctaaatttgcatcggtgtatgattccattgatgatgtggatctttggattggtggattagccgaacaggatgttaatggtggagtggttggtgagacaattagtgccatcattatcgagcaatttagtaatttacgggatggcgatcgcttttattttgaaaacgatcagtatctcaaggaacttaaaggcattcttgataagaatattgataaggttagtctcgctaatattatcgaagataactctgatgttcaaattgtgggtagtgcatttacagtcaataatcccatagttgtt

SEQ ID NO: 9 - DNA, 1977 bp, synthetic construct
  source 1..1977: mol_type = other DNA
atggatgataattacgaaaacaataattccattcagcaggcgtttgattttagcgagaatgaacaaacgcttctttccaatattaatgggcttggcgttgcccttgataacgatttttatgaaattgaagcgacagaaggcagtctggatatttttgtcgaattaacatttaaccataatgagggaaaccttgatctttttcttttcgattcgacaggcaacgaaattgcctcatctaacagtctcgatgacaatgaaattattgactttactgtagacaaggccggcacatattatattcaagtgacgagcggggatggcacgttttcgggcaacacatatgatctgttctgggatgacgtgatcgcagaaaatacatttcgtacgattaacggacttaataacaatttgcaaaatcccgaatttggatcagcgaccgagaaaggtaccaggtatacacaactacttagacttggaccagaagcttatcaggatgaactgagcgaaccgcgcggaggtggcttaaccacacccctggagttgccgtctgcccgagaggtgtctaacgctatcgccgatcagggcgaacaatccatcgcgaacgattttaaattgtcagattggttctggcaatggggacagtttattgatcacgacatcagcctcacagaagcggatacctcaggtgattcctttccgatcccagttccgacaggtgacccggatttcgatccattcggtactggaacgcagacaatcccgttgactcgctcaatttttgatcctgctacaggtacaacaaaccctcgtgaacagattaacgagataacggctttcttggatggttccatggtatacggcagcgacgaagcaacagcactgagccttagagcgaatgatggcactggaaaattggcaacatctatcggcccggatggggaaattctgctcccgacagactctgatgggaattttttggcaggtgatattagagttaacgaacaactaggtttaatctcagtacatacattgtttgttcgggaacacaatagactggcgcaaaaaaccgcggacgtcttagataacggcaaagggcgaaaggccaacaaacttaatgaactgttcgaagaatcaggcttgagccgaggagattttatctacgaatcagctaggcgtctggttggagcggaaattcaaacaatcacatataacgaatttcttccttttcttttagggaaaaatgtcctcgataagtacacagggtacgacgaaacggtcgatcctggcatattcacagaatttagcacaggcgtttttcgatttgggcatacgatgttatcaccacagctgttacaagtggaggaagatggctcgtatgaagcagttgctttaagagatgctttttttcagccaggcaaaattatggaagatggggttgattcactcctgaaaggactggagagccaacaggcacaagaagtggacaatcttctgattgacgacgttagaaacttcttatttgggcggccaggagcgggagggttcgacttagcatccttgaatatacaacgcgggcgcgagaatggagttgcagatattaacacgtttagaaacgccatcggtcttagcccgtatacagatttcgatgagcttaccggaggagattcagaattggcagcgaaattcgcttccgtctatgattcgattgatgatgtagacttgtggataggaggccttgctgaacaggatgtaaatggcggtgttgtgggggaaacaatctcagccattattatcgaacaatttagcaatctccgcgacggcgaccgtttctatttcgaaaatgatcaataccttaaagagttaaagggaattcttgataaaaacattgataaagttagcctcgctaacatcattgaagataactccgatgtgcaaattgtggggtccgcgttcacagtcaacaatccgattgtagtg

SEQ ID NO: 10 - protein, 659 aa, synthetic construct
MDDNYEKNNRIQKAFNLKKNEQTLLSDIDGLGIALDDDFYKIKATKGSLDIFVELTFNHNEGNLDLFLFDSKRNEIASSDSLDDNEIIDFTVDKAGTYYIQVTSGDGTFSGNTYDLLWDDVIGENTFRTINGLNNNLQNPEFGSATEKGTRYTQLLRLGPEAYEDGLSEPRGGGLTTPLELPSPRAVSNAIADQGEESIVNDFKLSDWFWQWGQFIDHDIDLTEADSSGDSFPIPVPTGDPDFDPSGTGTQIIPLTRSIFDPATGTTNPREQVNEITTFLDASMVYGSDEATALSLRANDGTGKLATSIGPDGEILLPTDGAGNFIAGDIRVNEQLGLTSVHTLFVREHNRLAQKTADVLDDGNGRKADKLNELFEESGLSRGDFIYESARRLVGAKIQTITYNEFLPLLLGKDALAEYTGYDETVEPGIFTEFSTGVFRFGHTMLSPQLLQVEEDGSYEAVALRDAFFQPSKIMEDGVDSLLKGLESQQAQAVDNFLIDDVRNFLFGPPGAGGFDLASLNIQRGRENGVADINTVRNAIGLSSYTDFDELTGGNSELAAKFASVYDSIDDVDLWIGGLAEQDVNGGVVGETISAIIIQQFTNLRDGDRFYFENDPYFQELEGIIDKNIDKVSLADIIEDNSDVKIVASAFTVNNPIVV

SEQ ID NO: 11 - protein, 659 aa, synthetic construct
MDDNYEKNNRIQQAFDFSENEQTLLSDINGLGVALDDDLYKIEATEGSLDIFVELTFNHNEGNLDLFLLDSTGNEIASSDSLDDNEIIDFTVDKAGTYYIQVTSGDGTFSGNTYDLLWDDVIGENTFRTINGLNNNLQNPEFGSATEKGTRYTQLLRLGPEAYEDGLSEPRGGGLTTPLELPSARAVSNAIADQGEESIVNDFKLSDWFWQWGQFIDHDIDLTEADSSGDSFPIQVPTGDPDFDPFGTGTQTIPLTRSIFDPATGTTNPREQINEITAFLDGSMVYGSDEATALSLRADDGTGKLATSIGPDGEILLPTDSDGNFLAGDIRVNEQLGLISVHTLFVREHNRLADEITDVLDNGNGSKADKLNELFEESGLSRGDFIYESARRLVGAKIQTITYNEFLPLLLGKDALGEYTGYDETLEPGIFTEFSTGVFRFGHTMLSPQLLQVEEDGSYEAVALRDAFFQPSKIMEDGVDSLLKGLESQQAQAVDNFLIDDVRNFLFGPPGAGGFDLASLNIQRGRENGVADINTVRNAIGLSSYTDFDELTGGNSELAAKFASVYDSIDDVDLWIGGLAEQDINGGVVGETISAIIIKQFTNLRDGDRFYVKNDPYLKELEGIIDKNLDNVSLADIIEDNSDVKIVASAFTVNNPIVV

SEQ ID NO: 12 - protein, 661 aa, synthetic construct
MQNNGNGNGNGNGNGSSKGSGNDDVYENNNSRRQAYDLTSLEQTPLSEIQGLAIAKNPDWYKIQVSPGTTSLSVDLQFTHADGNIDLFLHNANGNEIASSTSQTNNESINFDSPTAGVYYIKVKSIGKPGNSYDLVWDDIVPIEFRSIEGLNNNLVNPDWGTPDSQLIRLSESAYNDEISEPRGGDPSSLVSPREVSNTIFDQSESIPNETGVSDWFWQWGQFIDHDMDLTPGTSGESFNISVPLGDPSFDPFNSGTQEIPLTRSIYDFDTGIDSPREQINEITAYIDGSNVYGSDSERAEALRTNDGTGKLKTSVSESGEVLLPFNTDGLDNDNPFGIANDSIFVAGDVRANEQVGLTATHTLFVREHNRLADDIATRLDNGDAELLDLFAESGLSEGDFIYESARRIVGAEIQAITYNEFVPLLVGSNALDGYDGYNVTVDSGISNEFSTAAFRFGHTMLSPTLQNGTNEGLSLRDTFFNPDLVVEGGVDSLLLGLASQEAQEVDTQVIDDVRNFLFGAPGSGGLDLVSLNIQRGRDHGLPSYTEVREELGLDPITNFGEITSDPIVQAQLESAYTDVDNIDLWVGGLAEDHVNGSLFGETFQVIVVDQFTRLRDGDRFYYENDNLLSVLAPDVAETTLSDVIVANSAISSIQSNAFLV

SEQ ID NO: 13 - DNA, 1638 bp, synthetic construct
  source 1..1638: mol_type = other DNA
atgggtgtctactatattaaagtgaagagcattggtaaaccgggaaactcatatgaccttgtatgggatgatatcgttcctattgagtttcggtctattgaagggctgaacaacaatttggtcaatccggactggggcacaccggactcacagcttatccgtctgagcgaatcagcatacaacgacgaaattagcgagcctcgcggcggcgatccatcttctttagttagccctcgggaagtctcaaacacaattttcgatcagagcgaatcaatccctaatgagacgggcgtatctgactggttttggcaatggggccagtttatcgatcatgacatggatttgaccccgggaacatctggtgaatcatttaatatcagcgtgccactgggtgatccatcatttgacccgtttaatagcggaacccaagaaatcccgctgaccagatcaatctatgattttgatactggaattgattctccgcgtgaacaaatcaatgagatcacggcgtatattgacggatctaatgtgtatggaagcgattcagagcgcgccgaagctttgagaacgaatgatgggacaggaaaactgaagacgtctgtaagcgaatctggtgaagtcctgttaccgttcaacacagatggacttgataatgacaatccattcggaattgcaaacgattcaatttttgtagctggcgacgttcgggcgaatgaacaagttgggttaactgccacacatacattatttgttcgggaacataaccgtctggccgatgatatcgcgacccgcctggataatggtgatgcggaattgttagacctttttgcagagagcggactgtcagaaggcgatttcatctacgaaagcgctagacgcatcgttggggcagagattcaagcaattacgtacaatgaattcgttccgctgcttgtaggatcaaacgctcttgacggatatgacggctataatgtaacagtagatagcgggattagcaacgaattttctacggcagcctttagatttggacacactatgctgagccctacgcttcaaaatgggacgaatgaaggtctgagcctgcgcgatacctttttcaatccggatttagtggtcgaaggcggcgtagattctttgttattggggcttgcatctcaagaagctcaggaagtcgacactcaagtgattgatgatgtgcgtaactttttatttggtgcgcctggttctggtggccttgatcttgttagcttaaacatccagcgtggccgggatcatgggttgccgtcatatactgaagttagagaagagctgggattagatccgattacaaatttcggcgagatcacaagcgatccaattgtccaggcccaacttgagtcagcttatacagacgtcgacaatattgatttgtgggttggcggcttagcagaagaccacgtcaacggaagcttgtttggcgagacatttcaggtgattgtcgtggaccagtttactcgccttagagacggcgatagattctactatgagaacgataatttactttcagtgcttgcgcctgacgttgcggaaacgacattgtctgatgtgattgtggccaacagcgctatctcttcaatccagtcaaatgcgttcctggtc

SEQ ID NO: 14 - DNA, 20 bp, synthetic construct
  source 1..20: mol_type = other DNA
aaactgcggccggtgcacat

SEQ ID NO: 15 - DNA, 55 bp, synthetic construct
  source 1..55: mol_type = other DNA
ttttctgcagttaatggtggtggtgatgatggaccaggaacgcatttgactggat

SEQ ID NO: 16 - protein, 612 aa, synthetic construct
DTTLTNVTDPSLDLTALSWEVGCGAPVPLVKCDENSPYRTITGDCNNRRSPALGAANRALARWLPAEYEDGLALPFGWTQRKTRNGFRVPLAREVSNKIVGYLDEEGVLDQNRSLLFMQWGQIVDHDLDFAPETELGSNEHSKTQCEEYCIQGDNCFPIMFPKNDPKLKTQGKCMPFFRAGFVCPTPPYQSLAREQINAVTSFLDASLVYGSEPSLASRLRNLSSPLGLMAVNQEAWDHGLAYLPFNNKKPSPCEFINTTARVPCFLAGDFRASEQILLATAHTLLLREHNRLARELKKLNPHWNGEKLYQEARKILGAFIQIITFRDYLPIVLGSEMQKWIPPYQGYNNSVDPRISNVFTFAFRFGHMEVPSTVSRLDENYQPWGPEAELPLHTLFFNTWRIIKDGGIDPLVRGLLAKKSKLMNQDKMVTSELRNKLFQPTHKIHGFDLAAINLQRCRDHGMPGYNSWRGFCGLSQPKTLKGLQTVLKNKILAKKLMDLYKTPDNIDIWIGGNAEPMVERGRVGPLLACLLGRQFQQIRDGDRFWWENPGVFTEKQRDSLQKVSFSRLICDNTHITKVPLHAFQANNYPHDFVDCSTVDKLDLSPWASREN

SEQ ID NO: 17 - protein, 712 aa, synthetic construct
MWVCLQLPVFLASVTLFEVAASDTIAQAASTTTISDAVSKVKIQVNKAFLDSRTRLKTTLSSEAPTTQQLSEYFKHAKGRTRTAIRNGQVWEESLKRLRRDTTLTNVTDPSLDLTALSWEVGCGAPVPLVKCDENSPYRTITGDCNNRRSPALGAANRALARWLPAEYEDGLALPFGWTQRKTRNGFRVPLAREVSNKIVGYLDEEGVLDQNRSLLFMQWGQIVDHDLDFAPETELGSNEHSKTQCEEYCIQGDNCFPIMFPKNDPKLKTQGKCMPFFRAGFVCPTPPYQSLAREQINAVTSFLDASLVYGSEPSLASRLRNLSSPLGLMAVNQEAWDHGLAYLPFNNKKPSPCEFINTTARVPCFLAGDFRASEQILLATAHTLLLREHNRLARELKKLNPHWNGEKLYQEARKILGAFIQIITFRDYLPIVLGSEMQKWIPPYQGYNNSVDPRISNVFTFAFRFGHMEVPSTVSRLDENYQPWGPEAELPLHTLFFNTWRIIKDGGIDPLVRGLLAKKSKLMNQDKMVTSELRNKLFQPTHKIHGFDLAAINLQRCRDHGMPGYNSWRGFCGLSQPKTLKGLQTVLKNKILAKKLMDLYKTPDNIDIWIGGNAEPMVERGRVGPLLACLLGRQFQQIRDGDRFWWENPGVFTEKQRDSLQKVSFSRLICDNTHITKVPLHAFQANNYPHDFVDCSTVDKLDLSPWASREN

SEQ ID NO: 18 - protein, 543 aa, synthetic construct
FWDDVIAENTFRTINGLNNNLQNPEFGSATEKGTRYTQLLRLGPEAYQDELSEPRGGGLTTPLELPSAREVSNAIADQGEQSIANDFKLSDWFWQWGQFIDHDISLTEADTSGDSFPIPVPTGDPDFDPFGTGTQTIPLTRSIFDPATGTTNPREQINEITAFLDGSMVYGSDEATALSLRANDGTGKLATSIGPDGEILLPTDSDGNFLAGDIRVNEQLGLISVHTLFVREHNRLAQKTADVLDNGKGRKANKLNELFEESGLSRGDFIYESARRLVGAEIQTITYNEFLPFLLGKNVLDKYTGYDETVDPGIFTEFSTGVFRFGHTMLSPQLLQVEEDGSYEAVALRDAFFQPGKIMEDGVDSLLKGLESQQAQEVDNLLIDDVRNFLFGRPGAGGFDLASLNIQRGRENGVADINTFRNAIGLSPYTDFDELTGGDSELAAKFASVYDSIDDVDLWIGGLAEQDVNGGVVGETISAIIIEQFSNLRDGDRFYFENDQYLKELKGILDKNIDKVSLANIIEDNSDVQIVGSAFTVNNPIVV

SEQ ID NO: 19 - DNA, 1629 bp, synthetic construct
  source 1..1629: mol_type = other DNA
ttctgggatgacgtgatcgcagaaaatacatttcgtacgattaacggacttaataacaatttgcaaaatcccgaatttggatcagcgaccgagaaaggtaccaggtatacacaactacttagacttggaccagaagcttatcaggatgaactgagcgaaccgcgcggaggtggcttaaccacacccctggagttgccgtctgcccgagaggtgtctaacgctatcgccgatcagggcgaacaatccatcgcgaacgattttaaattgtcagattggttctggcaatggggacagtttattgatcacgacatcagcctcacagaagcggatacctcaggtgattcctttccgatcccagttccgacaggtgacccggatttcgatccattcggtactggaacgcagacaatcccgttgactcgctcaatttttgatcctgctacaggtacaacaaaccctcgtgaacagattaacgagataacggctttcttggatggttccatggtatacggcagcgacgaagcaacagcactgagccttagagcgaatgatggcactggaaaattggcaacatctatcggcccggatggggaaattctgctcccgacagactctgatgggaattttttggcaggtgatattagagttaacgaacaactaggtttaatctcagtacatacattgtttgttcgggaacacaatagactggcgcaaaaaaccgcggacgtcttagataacggcaaagggcgaaaggccaacaaacttaatgaactgttcgaagaatcaggcttgagccgaggagattttatctacgaatcagctaggcgtctggttggagcggaaattcaaacaatcacatataacgaatttcttccttttcttttagggaaaaatgtcctcgataagtacacagggtacgacgaaacggtcgatcctggcatattcacagaatttagcacaggcgtttttcgatttgggcatacgatgttatcaccacagctgttacaagtggaggaagatggctcgtatgaagcagttgctttaagagatgctttttttcagccaggcaaaattatggaagatggggttgattcactcctgaaaggactggagagccaacaggcacaagaagtggacaatcttctgattgacgacgttagaaacttcttatttgggcggccaggagcgggagggttcgacttagcatccttgaatatacaacgcgggcgcgagaatggagttgcagatattaacacgtttagaaacgccatcggtcttagcccgtatacagatttcgatgagcttaccggaggagattcagaattggcagcgaaattcgcttccgtctatgattcgattgatgatgtagacttgtggataggaggccttgctgaacaggatgtaaatggcggtgttgtgggggaaacaatctcagccattattatcgaacaatttagcaatctccgcgacggcgaccgtttctatttcgaaaatgatcaataccttaaagagttaaagggaattcttgataaaaacattgataaagttagcctcgctaacatcattgaagataactccgatgtgcaaattgtggggtccgcgttcacagtcaacaatccgattgtagtg

SEQ ID NO: 20 - DNA, 44 bp, synthetic construct
  source 1..44: mol_type = other DNA
tcaggctgcggccggtgcacatatgttctgggatgacgtgatcg

SEQ ID NO: 21 - DNA, 1980 bp, synthetic construct
  source 1..1980: mol_type = other DNA
atggacgacaattacgagaaaaataatcggatacaaaaagccttcaatctgaaaaaaaacgagcagacgttactctcagatattgatggattgggaatcgctctggatgacgatttctacaagatcaaagcgacgaagggcagcttagatatctttgttgaattaacttttaatcataatgaaggcaatcttgacttatttctttttgactcaaagcgaaacgagattgcatcttctgactcattagacgacaacgaaatcatcgattttactgttgataaagcgggtacatactacatccaggttacatctggggatggcacattttcgggtaacacatacgacttgctgtgggacgatgtaataggcgaaaatacttttcggacgattaatggcttgaacaataatttacagaatccggaatttggatctgccacagaaaaagggactcgctatactcagctcttgcggctggggccagaggcttacgaagacggtcttagcgagccgcggggcggcggtttgacgacaccgttagaactcccaagcccgagggcagtgtcgaatgcgatagcagaccagggagaggagtctatcgtgaatgattttaaactttcagattggttttggcaatggggacaatttatcgaccatgatattgatttaacagaagcggattctagcggagactcgttccctatccctgtacccacaggagatccggactttgatcctagcgggacgggcactcaaatcattccgctgactcgctctatattcgacccggcaaccggcacaacgaaccctcgggaacaggtcaatgagatcaccacgtttcttgacgcatccatggtttatggctcagatgaagccacagcgctgtcgttaagagcaaacgacggtacgggcaaattggctacctcgataggacctgacggtgaaatccttctccctacggatggtgccggcaactttatagctggggatatccgggtcaacgagcaattaggtttgacgtctgttcacacgttatttgtccgggagcataataggctcgcgcaaaaaactgctgacgttctcgatgacggtaatggacgcaaagcagataaactgaacgaacttttcgaagaatcaggccttagccgaggcgacttcatatacgagtcagcgcggcgtctcgtgggcgccaaaatccaaacaattacgtataatgaatttctcccccttttactgggcaaagatgccttggctgaatatacaggctacgatgagacagtggaaccgggaatttttacagaattcagcacaggagtattccgctttggacacaccatgttatcaccgcaactccttcaagtcgaagaagatgggtcgtacgaagcggtcgccctgcgtgatgccttcttccaaccttcaaagattatggaagatggtgtcgatagcctgttaaaaggtcttgaaagccaacaagcacaggcggttgacaactttttaatcgatgatgtgagaaacttcctttttggtccgcctggagccgggggattcgatttagcctctttaaacatccagcggggaagagaaaatggggtggctgatatcaacactgtacgaaacgcgattggattgtcaagctataccgactttgatgagttaacaggcggtaactctgagttggctgcgaaatttgcgagcgtttatgatagtatcgatgacgtagacttatggatcggcggtctggctgagcaggatgtcaatggcggcgtggtaggagagacgatatcggcgattatcatccagcagttcacaaatctcagagatggcgatcggttttattttgaaaacgacccatattttcaagaactggaaggtatcatcgacaagaatattgacaaggtctccttagctgatatcatcgaagataacagcgacgtcaagatcgtagctagcgcttttacggttaataacccgattgtcgtctaa

SEQ ID NO: 22 - DNA, 45 bp, synthetic construct
  source 1..45: mol_type = other DNA
tcaggctgcggccggtgcacatatgctgtgggacgatgtaatagg

SEQ ID NO: 23 - DNA, 53 bp, synthetic construct
  source 1..53: mol_type = other DNA
cagttaatggtggtggtgatgatggacgacaatcgggttattaaccgtaaaag

SEQ ID NO: 24 - DNA, 1629 bp, synthetic construct
  source 1..1629: mol_type = other DNA
ctgtgggacgatgtaataggcgaaaatacttttcggacgattaatggcttgaacaataatttacagaatccggaatttggatctgccacagaaaaagggactcgctatactcagctcttgcggctggggccagaggcttacgaagacggtcttagcgagccgcggggcggcggtttgacgacaccgttagaactcccaagcccgagggcagtgtcgaatgcgatagcagaccagggagaggagtctatcgtgaatgattttaaactttcagattggttttggcaatggggacaatttatcgaccatgatattgatttaacagaagcggattctagcggagactcgttccctatccctgtacccacaggagatccggactttgatcctagcgggacgggcactcaaatcattccgctgactcgctctatattcgacccggcaaccggcacaacgaaccctcgggaacaggtcaatgagatcaccacgtttcttgacgcatccatggtttatggctcagatgaagccacagcgctgtcgttaagagcaaacgacggtacgggcaaattggctacctcgataggacctgacggtgaaatccttctccctacggatggtgccggcaactttatagctggggatatccgggtcaacgagcaattaggtttgacgtctgttcacacgttatttgtccgggagcataataggctcgcgcaaaaaactgctgacgttctcgatgacggtaatggacgcaaagcagataaactgaacgaacttttcgaagaatcaggccttagccgaggcgacttcatatacgagtcagcgcggcgtctcgtgggcgccaaaatccaaacaattacgtataatgaatttctcccccttttactgggcaaagatgccttggctgaatatacaggctacgatgagacagtggaaccgggaatttttacagaattcagcacaggagtattccgctttggacacaccatgttatcaccgcaactccttcaagtcgaagaagatgggtcgtacgaagcggtcgccctgcgtgatgccttcttccaaccttcaaagattatggaagatggtgtcgatagcctgttaaaaggtcttgaaagccaacaagcacaggcggttgacaactttttaatcgatgatgtgagaaacttcctttttggtccgcctggagccgggggattcgatttagcctctttaaacatccagcggggaagagaaaatggggtggctgatatcaacactgtacgaaacgcgattggattgtcaagctataccgactttgatgagttaacaggcggtaactctgagttggctgcgaaatttgcgagcgtttatgatagtatcgatgacgtagacttatggatcggcggtctggctgagcaggatgtcaatggcggcgtggtaggagagacgatatcggcgattatcatccagcagttcacaaatctcagagatggcgatcggttttattttgaaaacgacccatattttcaagaactggaaggtatcatcgacaagaatattgacaaggtctccttagctgatatcatcgaagataacagcgacgtcaagatcgtagctagcgcttttacggttaataacccgattgtcgtc

SEQ ID NO: 25 - protein, 543 aa, synthetic construct
LWDDVIGENTFRTINGLNNNLQNPEFGSATEKGTRYTQLLRLGPEAYEDGLSEPRGGGLTTPLELPSARAVSNAIADQGEESIVNDFKLSDWFWQWGQFIDHDIDLTEADSSGDSFPIQVPTGDPDFDPFGTGTQTIPLTRSIFDPATGTTNPREQINEITAFLDGSMVYGSDEATALSLRADDGTGKLATSIGPDGEILLPTDSDGNFLAGDIRVNEQLGLISVHTLFVREHNRLADEITDVLDNGNGSKADKLNELFEESGLSRGDFIYESARRLVGAKIQTITYNEFLPLLLGKDALGEYTGYDETLEPGIFTEFSTGVFRFGHTMLSPQLLQVEEDGSYEAVALRDAFFQPSKIMEDGVDSLLKGLESQQAQAVDNFLIDDVRNFLFGPPGAGGFDLASLNIQRGRENGVADINTVRNAIGLSSYTDFDELTGGNSELAAKFASVYDSIDDVDLWIGGLAEQDINGGVVGETISAIIIKQFTNLRDGDRFYVKNDPYLKELEGIIDKNLDNVSLADIIEDNSDVKIVASAFTVNNPIVV

SEQ ID NO: 26 - protein, 544 aa, synthetic construct
MFWDDVIAENTFRTINGLNNNLQNPEFGSATEKGTRYTQLLRLGPEAYQDELSEPRGGGLTTPLELPSAREVSNAIADQGEQSIANDFKLSDWFWQWGQFIDHDISLTEADTSGDSFPIPVPTGDPDFDPFGTGTQTIPLTRSIFDPATGTTNPREQINEITAFLDGSMVYGSDEATALSLRANDGTGKLATSIGPDGEILLPTDSDGNFLAGDIRVNEQLGLISVHTLFVREHNRLAQKTADVLDNGKGRKANKLNELFEESGLSRGDFIYESARRLVGAEIQTITYNEFLPFLLGKNVLDKYTGYDETVDPGIFTEFSTGVFRFGHTMLSPQLLQVEEDGSYEAVALRDAFFQPGKIMEDGVDSLLKGLESQQAQEVDNLLIDDVRNFLFGRPGAGGFDLASLNIQRGRENGVADINTFRNAIGLSPYTDFDELTGGDSELAAKFASVYDSIDDVDLWIGGLAEQDVNGGVVGETISAIIIEQFSNLRDGDRFYFENDQYLKELKGILDKNIDKVSLANIIEDNSDVQIVGSAFTVNNPIVV

SEQ ID NO: 27 - protein, 544 aa, synthetic construct
MLWDDVIGENTFRTINGLNNNLQNPEFGSATEKGTRYTQLLRLGPEAYEDGLSEPRGGGLTTPLELPSARAVSNAIADQGEESIVNDFKLSDWFWQWGQFIDHDIDLTEADSSGDSFPIQVPTGDPDFDPFGTGTQTIPLTRSIFDPATGTTNPREQINEITAFLDGSMVYGSDEATALSLRADDGTGKLATSIGPDGEILLPTDSDGNFLAGDIRVNEQLGLISVHTLFVREHNRLADEITDVLDNGNGSKADKLNELFEESGLSRGDFIYESARRLVGAKIQTITYNEFLPLLLGKDALGEYTGYDETLEPGIFTEFSTGVFRFGHTMLSPQLLQVEEDGSYEAVALRDAFFQPSKIMEDGVDSLLKGLESQQAQAVDNFLIDDVRNFLFGPPGAGGFDLASLNIQRGRENGVADINTVRNAIGLSSYTDFDELTGGNSELAAKFASVYDSIDDVDLWIGGLAEQDINGGVVGETISAIIIKQFTNLRDGDRFYVKNDPYLKELEGIIDKNLDNVSLADIIEDNSDVKIVASAFTVNNPIVV

SEQ ID NO: 28 - DNA, 52 bp, synthetic construct
  source 1..52: mol_type = other DNA
ctgcggccggtgcacatatggacgacaattacgagaaaaataatcggataca